European Patent Application EP 4 512 904 A2, published February 26, 2025. Title: TREATMENT METHODS FOR FIBROSIS TARGETING SMOC2. Applicant: The Brigham and Women's Hospital, Inc. Application WO PCT/US2017/018753, filed February 21, 2017. The sequence listing filed with the application follows.

SEQUENCE LISTING (19 sequences)

SEQ ID NO: 1 - DNA, 20 bp, synthetic construct
  misc_feature 1..20: note = Wild type F primer
  source 1..20: mol_type = other DNA
tccttctccagcaccaagtc

SEQ ID NO: 2 - DNA, 20 bp, synthetic construct
  misc_feature 1..20: note = Wild type R primer
  source 1..20: mol_type = other DNA
tgatccaaaagtgcctcctc

SEQ ID NO: 3 - DNA, 20 bp, synthetic construct
  misc_feature 1..20: note = KO F primer
  source 1..20: mol_type = other DNA
cggtcgctaccattaccagt

SEQ ID NO: 4 - DNA, 24 bp, synthetic construct
  misc_feature 1..24: note = KO R primer
  source 1..24: mol_type = other DNA
catgctctgagaaataattaccaa

SEQ ID NO: 5 - DNA, 20 bp, synthetic construct
  misc_feature 1..20: note = Transgenic F primer
  source 1..20: mol_type = other DNA
tgacagcagcagcggcagtt

SEQ ID NO: 6 - DNA, 19 bp, synthetic construct
  misc_feature 1..19: note = Transgenic R primer
  source 1..19: mol_type = other DNA
tagcggctgaagcactgca

SEQ ID NO: 7 - DNA, 21 bp, synthetic construct
  misc_feature 1..21: note = aSMA F primer
  source 1..21: mol_type = other DNA
gtcccagacatcagggagtaa

SEQ ID NO: 8 - DNA, 21 bp, synthetic construct
  misc_feature 1..21: note = aSMA R primer
  source 1..21: mol_type = other DNA
tcggatacttcagcgtcagga

SEQ ID NO: 9 - DNA, 21 bp, synthetic construct
  misc_feature 1..21: note = Fibronectin F primer
  source 1..21: mol_type = other DNA
atgtggacccctcctgatagt

SEQ ID NO: 10 - DNA, 21 bp, synthetic construct
  misc_feature 1..21: note = Fibronectin R primer
  source 1..21: mol_type = other DNA
gcccagtgatttcagcaaagg

SEQ ID NO: 11 - DNA, 20 bp, synthetic construct
  misc_feature 1..20: note = Smoc2 F primer
  source 1..20: mol_type = other DNA
ccgtacaagaactgatgggc

SEQ ID NO: 12 - DNA, 20 bp, synthetic construct
  misc_feature 1..20: note = Smoc2 R primer
  source 1..20: mol_type = other DNA
ctttcagcatgacctctggg

SEQ ID NO: 13 - DNA, 20 bp, synthetic construct
  misc_feature 1..20: note = Col1a1 F primer
  source 1..20: mol_type = other DNA
tgactggaagagcggagagt

SEQ ID NO: 14 - DNA, 20 bp, synthetic construct
  misc_feature 1..20: note = Col1a1 R primer
  source 1..20: mol_type = other DNA
gttcgggctgatgtaccagt

SEQ ID NO: 15 - DNA, 22 bp, synthetic construct
  misc_feature 1..22: note = GAPDH F primer
  source 1..22: mol_type = other DNA
attgccctcaacgaccactttg

SEQ ID NO: 16 - DNA, 24 bp, synthetic construct
  misc_feature 1..24: note = GADPH R primer
  source 1..24: mol_type = other DNA
tctctcttcctcttgtgctcttgc

SEQ ID NO: 17 - RNA, 18 nt, synthetic construct
  misc_feature 1..18: note = siRNA target sequence
  source 1..18: mol_type = other RNA
tctgaactctgaatttaa

SEQ ID NO: 18 - RNA, 21 nt, synthetic construct
  misc_feature 1..21: note = SMOC2 siRNA Sense
  source 1..21: mol_type = other RNA
ttctgaactctgaatttaatt

SEQ ID NO: 19 - RNA, 21 nt, synthetic construct
  misc_feature 1..21: note = SMOC2 siRNA Antisense
  source 1..21: mol_type = other RNA
ttaaattcagagttcagaatt